European Patent Application EP 4 223 269 A2, published August 9, 2023. Title: USES OF ANTI-BCMA CHIMERIC ANTIGEN RECEPTORS. Applicant: Celgene Corporation. Application EP. The sequence listing filed with the application follows.

SEQUENCE LISTING (36 sequences)

SEQ ID NO: 1 - protein, 15 aa, Mus musculus
RASESVTILGSHLIH

SEQ ID NO: 2 - protein, 7 aa, Mus musculus
LASNVQT

SEQ ID NO: 3 - protein, 9 aa, Mus musculus
LQSRTIPRT

SEQ ID NO: 4 - protein, 5 aa, Mus musculus
DYSIN

SEQ ID NO: 5 - protein, 17 aa, Mus musculus
WINTETREPAYAYDFRG

SEQ ID NO: 6 - protein, 8 aa, Mus musculus
DYSYAMDY

SEQ ID NO: 7 - protein, 111 aa, Mus musculus
DIVLTQSPPSLAMSLGKRATISCRASESVTILGSHLIHWYQQKPGQPPTLLIQLASNVQTGVPARFSGSGSRTDFTLTIDPVEEDDVAVYYCLQSRTIPRTFGGGTKLEIK

SEQ ID NO: 8 - protein, 117 aa, Mus musculus
QIQLVQSGPELKKPGETVKISCKASGYTFTDYSINWVKRAPGKGLKWMGWINTETREPAYAYDFRGRFAFSLETSASTAYLQINNLKYEDTATYFCALDYSYAMDYWGQGTSVTVSS

SEQ ID NO: 9 - protein, 493 aa, synthetic construct
  REGION 1..493: note = anti-BCMA02 CAR
MALPVTALLLPLALLLHAARPDIVLTQSPPSLAMSLGKRATISCRASESVTILGSHLIHWYQQKPGQPPTLLIQLASNVQTGVPARFSGSGSRTDFTLTIDPVEEDDVAVYYCLQSRTIPRTFGGGTKLEIKGSTSGSGKPGSGEGSTKGQIQLVQSGPELKKPGETVKISCKASGYTFTDYSINWVKRAPGKGLKWMGWINTETREPAYAYDFRGRFAFSLETSASTAYLQINNLKYEDTATYFCALDYSYAMDYWGQGTSVTVSSAAATTTPAPRPPTPAPTIASQPLSLRPEACRPAAGGAVHTRGLDFACDIYIWAPLAGTCGVLLLSLVITLYCKRGRKKLLYIFKQPFMRPVQTTQEEDGCSCRFPEEEEGGCELRVKFSRSADAPAYQQGQNQLYNELNLGRREEYDVLDKRRGRDPEMGGKPRRKNPQEGLYNELQKDKMAEAYSEIGMKGERRRGKGHDGLYQGLSTATKDTYDALHMQALPPR

SEQ ID NO: 10 - DNA, 1485 bp, synthetic construct
  misc_feature 1..1485: note = anti-BCMA02 CAR
  source 1..1485: mol_type = other DNA
atggcactccccgtcaccgcccttctcttgcccctcgccctgctgctgcatgctgccaggcccgacattgtgctcactcagtcacctcccagcctggccatgagcctgggaaaaagggccaccatctcctgtagagccagtgagtccgtcacaatcttggggagccatcttattcactggtatcagcagaagcccgggcagcctccaacccttcttattcagctcgcgtcaaacgtccagacgggtgtacctgccagattttctggtagcgggtcccgcactgattttacactgaccatagatccagtggaagaagacgatgtggccgtgtattattgtctgcagagcagaacgattcctcgcacatttggtgggggtactaagctggagattaagggaagcacgtccggctcagggaagccgggctccggcgagggaagcacgaaggggcaaattcagctggtccagagcggacctgagctgaaaaaacccggcgagactgttaagatcagttgtaaagcatctggctataccttcaccgactacagcataaattgggtgaaacgggcccctggaaagggcctcaaatggatgggttggatcaataccgaaactagggagcctgcttatgcatatgacttccgcgggagattcgccttttcactcgagacatctgcctctactgcttacctccaaataaacaacctcaagtatgaagatacagccacttacttttgcgccctcgactatagttacgccatggactactggggacagggaacctccgttaccgtcagttccgcggccgcaaccacaacacctgctccaaggccccccacacccgctccaactatagccagccaaccattgagcctcagacctgaagcttgcaggcccgcagcaggaggcgccgtccatacgcgaggcctggacttcgcgtgtgatatttatatttgggcccctttggccggaacatgtggggtgttgcttctctcccttgtgatcactctgtattgtaagcgcgggagaaagaagctcctgtacatcttcaagcagccttttatgcgacctgtgcaaaccactcaggaagaagatgggtgttcatgccgcttccccgaggaggaagaaggagggtgtgaactgagggtgaaattttctagaagcgccgatgctcccgcatatcagcagggtcagaatcagctctacaatgaattgaatctcggcaggcgagaagagtacgatgttctggacaagagacggggcagggatcccgagatggggggaaagccccggagaaaaaatcctcaggaggggttgtacaatgagctgcagaaggacaagatggctgaagcctatagcgagatcggaatgaaaggcgaaagacgcagaggcaaggggcatgacggtctgtaccagggtctctctacagccaccaaggacacttatgatgcgttgcatatgcaagccttgccaccccgctaatga

SEQ ID NO: 11 - protein, 184 aa, Homo sapiens
MLQMAGQCSQNEYFDSLLHACIPCQLRCSSNTPPLTCQRYCNASVTNSVKGTNAILWTCLGLSLIISLAVFVLMFLLRKINSEPLKDEFKNTGSGLLGMANIDLEKSRTGDEIILPRGLEYTVEECTCEDCIKSKPKVDSDHCFPLPAMEEGATILVTTKTNDYCKSLPAALSATEIEKSISAR

SEQ ID NO: 12 - protein, 5 aa, synthetic construct
  REGION 1..5: note = Flexible peptide linker
DGGGS

SEQ ID NO: 13 - protein, 5 aa, synthetic construct
  REGION 1..5: note = Flexible peptide linker
TGEKP

SEQ ID NO: 14 - protein, 4 aa, synthetic construct
  REGION 1..4: note = Flexible peptide linker
GGRR

SEQ ID NO: 15 - protein, 5 aa, synthetic construct
  REGION 1..5: note = Flexible peptide linker
GGGGS

SEQ ID NO: 16 - protein, 14 aa, synthetic construct
  REGION 1..14: note = Flexible peptide linker
EGKSSGSGSESKVD

SEQ ID NO: 17 - protein, 18 aa, synthetic construct
  REGION 1..18: note = Flexible peptide linker
KESGSVSSEQLAQFRSLD

SEQ ID NO: 18 - protein, 8 aa, synthetic construct
  REGION 1..8: note = Flexible peptide linker
GGRRGGGS

SEQ ID NO: 19 - protein, 9 aa, synthetic construct
  REGION 1..9: note = Flexible peptide linker
LRQRDGERP

SEQ ID NO: 20 - protein, 12 aa, synthetic construct
  REGION 1..12: note = Flexible peptide linker
LRQKDGGGSERP

SEQ ID NO: 21 - protein, 16 aa, synthetic construct
  REGION 1..16: note = Flexible peptide linker
LRQKDGGGSGGGSERP

SEQ ID NO: 22 - protein, 18 aa, synthetic construct
  REGION 1..18: note = Flexible peptide linker
GSTSGSGKPGSGEGSTKG

SEQ ID NO: 23 - skipped

SEQ ID NO: 24 - protein, 7 aa, synthetic construct
  REGION 1..7: note = protease cleavage site
ENLYFQG

SEQ ID NO: 25 - protein, 7 aa, synthetic construct
  REGION 1..7: note = protease cleavage site
ENLYFQS

SEQ ID NO: 26 - protein, 19 aa, synthetic construct
  REGION 1..19: note = protease cleavage site
LLNFDLLKLAGDVESNPGP

SEQ ID NO: 27 - protein, 19 aa, synthetic construct
  REGION 1..19: note = protease cleavage site
TLNFDLLKLAGDVESNPGP

SEQ ID NO: 28 - protein, 14 aa, synthetic construct
  REGION 1..14: note = protease cleavage site
LLKLAGDVESNPGP

SEQ ID NO: 29 - protein, 17 aa, synthetic construct
  REGION 1..17: note = protease cleavage site
NFDLLKLAGDVESNPGP

SEQ ID NO: 30 - protein, 20 aa, synthetic construct
  REGION 1..20: note = protease cleavage site
QLLNFDLLKLAGDVESNPGP

SEQ ID NO: 31 - protein, 24 aa, synthetic construct
  REGION 1..24: note = protease cleavage site
APVKQTLNFDLLKLAGDVESNPGP

SEQ ID NO: 32 - protein, 40 aa, synthetic construct
  REGION 1..40: note = protease cleavage site
VTELLYRMKRAETYCPRPLLAIHPTEARHKQKIVAPVKQT

SEQ ID NO: 33 - protein, 18 aa, synthetic construct
  REGION 1..18: note = protease cleavage site
LNFDLLKLAGDVESNPGP

SEQ ID NO: 34 - protein, 40 aa, synthetic construct
  REGION 1..40: note = protease cleavage site
LLAIHPTEARHKQKIVAPVKQTLNFDLLKLAGDVESNPGP

SEQ ID NO: 35 - protein, 33 aa, synthetic construct
  REGION 1..33: note = protease cleavage site
EARHKQKIVAPVKQTLNFDLLKLAGDVESNPGP

SEQ ID NO: 36 - DNA, 7350 bp, synthetic construct
  misc_feature 1..7350: note = anti-BCMA02 CAR vector
  source 1..7350: mol_type = other DNA
tcgcgcgtttcggtgatgacggtgaaaacctctgacacatgcagctcccggagacggtcacagcttgtctgtaagcggatgccgggagcagacaagcccgtcagggcgcgtcagcgggtgttggcgggtgtcggggctggcttaactatgcggcatcagagcagattgtactgagagtgcaccatcatatgccagcctatggtgacattgattattgactagttattaatagtaatcaattacggggtcattagttcatagcccatatatggagttccgcgttacataacttacggtaaatggcccgcctggctgaccgcccaacgacccccgcccattgacgtcaataatgacgtatgttcccatagtaacgccaatagggactttccattgacgtcaatgggtggagtatttacggtaaactgcccacttggcagtacatcaagtgtatcatatgccaagtacgccccctattgacgtcaatgacggtaaatggcccgcctggcattatgcccagtacatgaccttatgggactttcctacttggcagtacatctacgtattagtcatcgctattaccatggtgatgcggttttggcagtacatcaatgggcgtggatagcggtttgactcacggggatttccaagtctccaccccattgacgtcaatgggagtttgttttggcaccaaaatcaacgggactttccaaaatgtcgtaacaactccgccccattgacgcaaatgggcggtaggcgtgtacggtgggaggtctatataagcagagctcgtttagtgaaccgggtctctctggttagaccagatctgagcctgggagctctctggctaactagggaacccactgcttaagcctcaataaagcttgccttgagtgctcaaagtagtgtgtgcccgtctgttgtgtgactctggtaactagagatccctcagacccttttagtcagtgtggaaaatctctagcagtggcgcccgaacagggacttgaaagcgaaagtaaagccagaggagatctctcgacgcaggactcggcttgctgaagcgcgcacggcaagaggcgaggggcggcgactggtgagtacgccaaaaattttgactagcggaggctagaaggagagagtagggtgcgagagcgtcggtattaagcgggggagaattagataaatgggaaaaaattcggttaaggccagggggaaagaaacaatataaactaaaacatatagttagggcaagcagggagctagaacgattcgcagttaatcctggccttttagagacatcagaaggctgtagacaaatactgggacagctacaaccatcccttcagacaggatcagaagaacttagatcattatataatacaatagcagtcctctattgtgtgcatcaaaggatagatgtaaaagacaccaaggaagccttagataagatagaggaagagcaaaacaaaagtaagaaaaaggcacagcaagcagcagctgacacaggaaacaacagccaggtcagccaaaattaccctatagtgcagaacctccaggggcaaatggtacatcaggccatatcacctagaactttaaattaagacagcagtacaaatggcagtattcatccacaattttaaaagaaaaggggggattggggggtacagtgcaggggaaagaatagtagacataatagcaacagacatacaaactaaagaattacaaaaacaaattacaaaaattcaaaattttcgggtttattacagggacagcagagatccagtttggaaaggaccagcaaagctcctctggaaaggtgaaggggcagtagtaatacaagataatagtgacataaaagtagtgccaagaagaaaagcaaagatcatcagggattatggaaaacagatggcaggtgatgattgtgtggcaagtagacaggatgaggattaacacatggaaaagattagtaaaacaccatagctctagagcgatcccgatcttcagacctggaggaggagatatgagggacaattggagaagtgaattatataaatataaagtagtaaaaattgaaccattaggagtagcacccaccaaggcaaagagaagagtggtgcagagagaaaaaagagcagtgggaataggagctttgttccttgggttcttgggagcagcaggaagcactatgggcgcagcgtcaatgacgctgacggtacaggccagacaattattgtctggtatagtgcagcagcagaacaatttgctgagggctattgaggcgcaacagcatctgttgcaactcacagtctggggcatcaagcagctccaggcaagaatcctggctgtggaaagatacctaaaggatcaacagctcctggggatttggggttgctctggaaaactcatttgcaccactgctgtgccttggaatgctagttggagtaataaatctctggaacagatttggaatcacacgacctggatggagtgggacagagaaattaacaattacacaagcttggtaggtttaagaatagtttttgctgtactttctatagtgaatagagttaggcagggatattcaccattatcgtttcagacccacctcccaaccccgaggggacccgacaggcccgaaggaatagaagaagaaggtggagagagagacagagacagatccattcgattagtgaacggatccatctcgacggaatgaaagaccccacctgtaggtttggcaagctaggatcaaggttaggaacagagagacagcagaatatgggccaaacaggatatctgtggtaagcagttcctgccccggctcagggccaagaacagttggaacagcagaatatgggccaaacaggatatctgtggtaagcagttcctgccccggctcagggccaagaacagatggtccccagatgcggtcccgccctcagcagtttctagagaaccatcagatgtttccagggtgccccaaggacctgaaatgaccctgtgccttatttgaactaaccaatcagttcgcttctcgcttctgttcgcgcgcttctgctccccgagctcaataaaagagcccacaacccctcactcggcgcgattcacctgacgcgtctacgccaccatggcactccccgtcaccgcccttctcttgcccctcgccctgctgctgcatgctgccaggcccgacattgtgctcactcagtcacctcccagcctggccatgagcctgggaaaaagggccaccatctcctgtagagccagtgagtccgtcacaatcttggggagccatcttattcactggtatcagcagaagcccgggcagcctccaacccttcttattcagctcgcgtcaaacgtccagacgggtgtacctgccagattttctggtagcgggtcccgcactgattttacactgaccatagatccagtggaagaagacgatgtggccgtgtattattgtctgcagagcagaacgattcctcgcacatttggtgggggtactaagctggagattaagggaagcacgtccggctcagggaagccgggctccggcgagggaagcacgaaggggcaaattcagctggtccagagcggacctgagctgaaaaaacccggcgagactgttaagatcagttgtaaagcatctggctataccttcaccgactacagcataaattgggtgaaacgggcccctggaaagggcctcaaatggatgggttggatcaataccgaaactagggagcctgcttatgcatatgacttccgcgggagattcgccttttcactcgagacatctgcctctactgcttacctccaaataaacaacctcaagtatgaagatacagccacttacttttgcgccctcgactatagttacgccatggactactggggacagggaacctccgttaccgtcagttccgcggccgcaaccacaacacctgctccaaggccccccacacccgctccaactatagccagccaaccattgagcctcagacctgaagcttgcaggcccgcagcaggaggcgccgtccatacgcgaggcctggacttcgcgtgtgatatttatatttgggcccctttggccggaacatgtggggtgttgcttctctcccttgtgatcactctgtattgtaagcgcgggagaaagaagctcctgtacatcttcaagcagccttttatgcgacctgtgcaaaccactcaggaagaagatgggtgttcatgccgcttccccgaggaggaagaaggagggtgtgaactgagggtgaaattttctagaagcgccgatgctcccgcatatcagcagggtcagaatcagctctacaatgaattgaatctcggcaggcgagaagagtacgatgttctggacaagagacggggcagggatcccgagatggggggaaagccccggagaaaaaatcctcaggaggggttgtacaatgagctgcagaaggacaagatggctgaagcctatagcgagatcggaatgaaaggcgaaagacgcagaggcaaggggcatgacggtctgtaccagggtctctctacagccaccaaggacacttatgatgcgttgcatatgcaagccttgccaccccgctaatgacaggtacctttaagaccaatgacttacaaggcagctgtagatcttagccactttttaaaagaaaaggggggactggaagggctaattcactcccaaagaagacaagatctgctttttgcctgtactgggtctctctggttagaccagatctgagcctgggagctctctggctaactagggaacccactgcttaagcctcaataaagcttgccttgagtgcttcaatgtgtgtgttggttttttgtgtgtcgaaattctagcgattctagcttggcgtaatcatggtcatagctgtttcctgtgtgaaattgttatccgctcacaattccacacaacatacgagccggaagcataaagtgtaaagcctggggtgcctaatgagtgagctaactcacattaattgcgttgcgctcactgcccgctttccagtcgggaaacctgtcgtgccagctgcattaatgaatcggccaacgcgcggggagaggcggtttgcgtattgggcgctcttccgcttcctcgctcactgactcgctgcgctcggtcgttcggctgcggcgagcggtatcagctcactcaaaggcggtaatacggttatccacagaatcaggggataacgcaggaaagaacatgtgagcaaaaggccagcaaaaggccaggaaccgtaaaaaggccgcgttgctggcgtttttccataggctccgcccccctgacgagcatcacaaaaatcgacgctcaagtcagaggtggcgaaacccgacaggactataaagataccaggcgtttccccctggaagctccctcgtgcgctctcctgttccgaccctgccgcttaccggatacctgtccgcctttctcccttcgggaagcgtggcgctttctcatagctcacgctgtaggtatctcagttcggtgtaggtcgttcgctccaagctgggctgtgtgcacgaaccccccgttcagcccgaccgctgcgccttatccggtaactatcgtcttgagtccaacccggtaagacacgacttatcgccactggcagcagccactggtaacaggattagcagagcgaggtatgtaggcggtgctacagagttcttgaagtggtggcctaactacggctacactagaagaacagtatttggtatctgcgctctgctgaagccagttaccttcggaaaaagagttggtagctcttgatccggcaaacaaaccaccgctggtagcggtggtttttttgtttgcaagcagcagattacgcgcagaaaaaaaggatctcaagaagatcctttgatcttttctacggggtctgacgctcagtggaacgaaaactcacgttaagggattttggtcatgagattatcaaaaaggatcttcacctagatccttttaaattaaaaatgaagttttaaatcaatctaaagtatatatgagtaaacttggtctgacagttaccaatgcttaatcagtgaggcacctatctcagcgatctgtctatttcgttcatccatagttgcctgactccccgtcgtgtagataactacgatacgggagggcttaccatctggccccagtgctgcaatgataccgcgagacccacgctcaccggctccagatttatcagcaataaaccagccagccggaagggccgagcgcagaagtggtcctgcaactttatccgcctccatccagtctattaattgttgccgggaagctagagtaagtagttcgccagttaatagtttgcgcaacgttgttgccattgctacaggcatcgtggtgtcacgctcgtcgtttggtatggcttcattcagctccggttcccaacgatcaaggcgagttacatgatcccccatgttgtgcaaaaaagcggttagctccttcggtcctccgatcgttgtcagaagtaagttggccgcagtgttatcactcatggttatggcagcactgcataattctcttactgtcatgccatccgtaagatgcttttctgtgactggtgagtactcaaccaagtcattctgagaatagtgtatgcggcgaccgagttgctcttgcccggcgtcaatacgggataataccgcgccacatagcagaactttaaaagtgctcatcattggaaaacgttcttcggggcgaaaactctcaaggatcttaccgctgttgagatccagttcgatgtaacccactcgtgcacccaactgatcttcagcatcttttactttcaccagcgtttctgggtgagcaaaaacaggaaggcaaaatgccgcaaaaaagggaataagggcgacacggaaatgttgaatactcatactcttcctttttcaatattattgaagcatttatcagggttattgtctcatgagcggatacatatttgaatgtatttagaaaaataaacaaataggggttccgcgcacatttccccgaaaagtgccacctgggactagctttttgcaaaagcctaggcctccaaaaaagcctcctcactacttctggaatagctcagaggccgaggcggcctcggcctctgcataaataaaaaaaattagtcagccatggggcggagaatgggcggaactgggcggagttaggggcgggatgggcggagttaggggcgggactatggttgctgactaattgagatgagcttgcatgccgacattgattattgactagtccctaagaaaccattcttatcatgacattaacctataaaaataggcgtatcacgaggccctttcgtc